European Patent Application EP 4 382 110 A1, published June 12, 2024. Title: Hairpin nucleic acid composition. Applicant: The University of Tokyo. The sequence listing filed with the application follows.

SEQUENCE LISTING (15 sequences)

SEQ ID NO: 1 - RNA, 22 nt, Homo sapiens
uagcuuaucagacugauguuga

SEQ ID NO: 2 - DNA, 46 bp, Artificial
  synthetic
tcaacatcagtctgataagctagggactttcctagcttatcagact

SEQ ID NO: 3 - DNA, 46 bp, Artificial
  synthetic
tagcttatcagactgatgttgaagtctgataagctaggaaagtccc

SEQ ID NO: 4 - DNA, 45 bp, Artificial
  synthetic
tcaacatcagtctgataagctagggactttcctagcttatcagac

SEQ ID NO: 5 - DNA, 45 bp, Artificial
  synthetic
tagcttatcagactgatgttgagtctgataagctaggaaagtccc

SEQ ID NO: 6 - DNA, 44 bp, Artificial
  synthetic
tcaacatcagtctgataagctagggactttcctagcttatcaga

SEQ ID NO: 7 - DNA, 44 bp, Artificial
  synthetic
tagcttatcagactgatgttgatctgataagctaggaaagtccc

SEQ ID NO: 8 - DNA, 46 bp, Artificial; identical to SEQ ID NO: 2
  synthetic
  misc_feature (21)..(21): FAM-T

SEQ ID NO: 9 - DNA, 46 bp, Artificial; identical to SEQ ID NO: 3
  synthetic
  misc_feature (46)..(46): C-TAMRA

SEQ ID NO: 10 - DNA, 46 bp, Artificial; identical to SEQ ID NO: 2
  synthetic
  misc_feature (1)..(9): internucleoside bonds are phosphorothioate bonds
  misc_feature (46)..(46): thymidine residue in which Cy5 is bound by C6 amino linker

SEQ ID NO: 11 - DNA, 46 bp, Artificial; identical to SEQ ID NO: 3
  synthetic
  misc_feature (25)..(25): thymidine residue replaced by a thymidine analog dT-FAM (3')
  misc_feature (36)..(46): internucleoside bonds are phosphorothioate bonds

SEQ ID NO: 12 - DNA, 24 bp, Artificial
  synthetic
acaggttacctccgaaactgaaga

SEQ ID NO: 13 - DNA, 25 bp, Artificial
  synthetic
ttagccatcagtcacttaaacagca

SEQ ID NO: 14 - protein, 522 aa, Homo sapiens
MQPWHGKAMQRASEAGATAPKASARNARGAPMDPTESPAAPEAALPKAGKFGPARKSGSRQKKSAPDTQERPPVRATGARAKKAPQRAQDTQPSDATSAPGAEGLEPPAAREPALSRAGSCRQRGARCSTKPRPPPGPWDVPSPGLPVSAPILVRRDAAPGASKLRAVLEKLKLSRDDISTAAGMVKGVVDHLLLRLKCDSAFRGVGLLNTGSYYEHVKISAPNEFDVMFKLEVPRIQLEEYSNTRAYYFVKFKRNPKENPLSQFLEGEILSASKMLSKFRKIIKEEINDIKDTDVIMKRKRGGSPAVTLLISEKISVDITLALESKSSWPASTQEGLRIQNWLSAKVRKQLRLKPFYLVPKHAKEGNGFQEETWRLSFSHIEKEILNNHGKSKTCCENKEEKCCRKDCLKLMKYLLEQLKERFKDKKHLDKFSSYHVKTAFFHVCTQNPQDSQWDRKDLGLCFDNCVTYFLQCLRTEKLENYFIPEFNLFSSNLIDKRSKEFLTKQIEYERNNEFPVFDEF

SEQ ID NO: 15 - protein, 435 aa, Homo sapiens
MSNGYSTDENFRYLISCFRARVKMYIQVEPVLDYLTFLPAEVKEQIQRTVATSGNMQAVELLLSTLEKGVWHLGWTREFVEALRRTGSPLAARYMNPELTDLPSPSFENAHDEYLQLLNLLQPTLVDKLLVRDVLDKCMEEELLTIEDRNRIAAAENNGNESGVRELLKRIVQKENWFSAFLNVLRQTGNNELVQELTGSDCSESNAEIENLSQVDGPQVEEQLLSTTVQPNLEKEVWGMENNSSESSFADSSVVSESDTSLAEGSVSCLDESLGHNSNMGSDSGTMGSDSDEENVAARASPEPELQLRPYQMEVAQPALEGKNIIICLPTGSGKTRVAVYIAKDHLDKKKKASEPGKVIVLVNKVLLVEQLFRKEFQPFLKKWYRVIGLSGDTQLKISFPEVVKSCDIIISTAQILENSLLNLENGEDAGVQLS